European Patent Application EP 4 674 967 A1, published January 7, 2026. Title: ENGINEERED DNA MOLECULE FOR CODING RNA. Applicant: RINUAGENE BIOTECHNOLOGY CO. , LTD. Application US. The sequence listing filed with the application follows.

SEQUENCE LISTING (26 sequences)

SEQ ID NO: 1 - DNA, 124 bp, synthetic construct
  source 1..124: mol_type = other DNA
aaaaaaaaaaaaaaaaaaaaaaaaaaaaaaaaaaaaaaaaaaaaaaaaaaaaaaaaaaaagaaaaaaaaaaaaaaaaaaagaaaaaaaaaaaaaaaaaaagaaaaaaaaaaaaaaaaaaagaaa

SEQ ID NO: 2 - DNA, 130 bp, synthetic construct
  source 1..130: mol_type = other DNA
aaaaaaacaaaaaaaaaaaaaaaaaagaaaaaaaaaaaaaaaaaaaaaaaaaaaaaaaaaaaaaaaaaaaaaaaaaaaaaaaaaaaaggaaaaaaacaaaaaaaaaaaaaaaaaagaaaaaaaaaaaaaa

SEQ ID NO: 3 - DNA, 123 bp, synthetic construct
  source 1..123: mol_type = other DNA
aaaaaaaaaaaaaaaaaaaaaaaaaaaaaaaaaaaaaaaaaaaaaaaaaaaaaaaaaaaagatatcaaaaaaaaaaaaaaaaaaagaaaaaaaaaaaaaaaaaaagaaaaaaaaaaaaaaaaa

SEQ ID NO: 4 - DNA, 125 bp, synthetic construct
  source 1..125: mol_type = other DNA
aaaaaaaaaaaaaaaaaaagaaaaaaaaaaaaaaaaaaagaaaaaaaaaaaaaaaaaaagatatcaaaaaaaaaaaaaaaaaaaaaaaaaaaaaaaaaaaaaaaaaaaaaaaaaaaaaaaaaaaa

SEQ ID NO: 5 - DNA, 126 bp, synthetic construct
  source 1..126: mol_type = other DNA
aaaaaaaaaaaaaaaaaaagaaaaaaaaaaaaaaaaaaagaaaaaaaaaaaaaaaaaaagatatcaaaaaaaaaaaaaaaaaaaaaaaaaaaaaaaaaaaaaaaaaaaaaaaaaaaaaaaaaaaag

SEQ ID NO: 6 - DNA, 125 bp, synthetic construct
  source 1..125: mol_type = other DNA
aaaaaaaaaaaaaaaaaaagaaaaaaaaaaaaaaaaaaagaaaaaaaaaaaaaaaaaaagtatacaaaaaaaaaaaaaaaaaaaaaaaaaaaaaaaaaaaaaaaaaaaaaaaaaaaaaaaaaaaa

SEQ ID NO: 7 - DNA, 131 bp, synthetic construct
  source 1..131: mol_type = other DNA
aaaaaaaaaaaaaaaaaaagaaaaaaaaaaaaaaaaaaagaaaaaaaaaaaaaaaaaaagatatcgtatacaaaaaaaaaaaaaaaaaaaaaaaaaaaaaaaaaaaaaaaaaaaaaaaaaaaaaaaaaaaa

SEQ ID NO: 8 - DNA, 125 bp, synthetic construct
  source 1..125: mol_type = other DNA
aaaaaaaaaaaaaaaaaaacaaaaaaaaaaaaaaaaaaacaaaaaaaaaaaaaaaaaaagatatcaaaaaaaaaaaaaaaaaaaaaaaaaaaaaaaaaaaaaaaaaaaaaaaaaaaaaaaaaaaa

SEQ ID NO: 9 - DNA, 125 bp, synthetic construct
  source 1..125: mol_type = other DNA
aaaaaaaaaaaaaaaaaaataaaaaaaaaaaaaaaaaaataaaaaaaaaaaaaaaaaaagatatcaaaaaaaaaaaaaaaaaaaaaaaaaaaaaaaaaaaaaaaaaaaaaaaaaaaaaaaaaaaa

SEQ ID NO: 10 - DNA, 125 bp, synthetic construct
  source 1..125: mol_type = other DNA
aaaaaaaaaaaaaaaaaaagaaaaaaaaaaaaaaaaaaagaaaaaaaaaaaaaaaaaaagaatctaaaaaaaaaaaaaaaaaaaaaaaaaaaaaaaaaaaaaaaaaaaaaaaaaaaaaaaaaaaa

SEQ ID NO: 11 - DNA, 130 bp, synthetic construct
  source 1..130: mol_type = other DNA
aaaaaaaaaaaaaaaaaaaaaaaaaaaaaaaaaaaaaaaaaaaaaaaaaaaaaaaaaaaagcatatgactaaaaaaaaaaaaaaaaaaaaaaaaaaaaaaaaaaaaaaaaaaaaaaaaaaaaaaaaaaaa

SEQ ID NO: 12 - DNA, 110 bp, synthetic construct
  source 1..110: mol_type = other DNA
aaaaaaaaaaaaaaaaaaaaaaaaaaaaaagcatatgactaaaaaaaaaaaaaaaaaaaaaaaaaaaaaaaaaaaaaaaaaaaaaaaaaaaaaaaaaaaaaaaaaaaaaa

SEQ ID NO: 13 - DNA, 121 bp, synthetic construct
  source 1..121: mol_type = other DNA
aaaaaaaaaaaaaaaaaaaaaaaaaaaaaaaaaaaaaaaaaaaaaaaaaaaaaaaaaaaagaaaaaaaaaaaaaaaaaaaaaaaaaaaaaaaaaaaaaaaaaaaaaaaaaaaaaaaaaaaa

SEQ ID NO: 14 - DNA, 126 bp, synthetic construct
  source 1..126: mol_type = other DNA
aaaaaaaaaaaaaaaaaaaaaaaaaaaaaaaaaaaaaaaaaaaaaaaaaaaaaaaaaaaaatgcataaaaaaaaaaaaaaaaaaaaaaaaaaaaaaaaaaaaaaaaaaaaaaaaaaaaaaaaaaaa

SEQ ID NO: 15-17 - skipped (3 entries)

SEQ ID NO: 18 - DNA, 10 bp, synthetic construct
  source 1..10: mol_type = other DNA
gcatatgact

SEQ ID NO: 19 - DNA, 12 bp, synthetic construct
  source 1..12: mol_type = other DNA
gatatcgtatac

SEQ ID NO: 20 - DNA, 213 bp, synthetic construct
  source 1..213: mol_type = other DNA
ctcgctttcttgctgtccaatttctattaaaggttcctttgttccctaagtccaactactaaactgggggatattatgaagggccttgagcatctggattctgcctgctcgctttcttgctgtccaatttctattaaaggttcctttgttccctaagtccaactactaaactgggggatattatgaagggccttgagcatctggattctgcct

SEQ ID NO: 21 - DNA, 50 bp, synthetic construct
  source 1..50: mol_type = other DNA
acatttgcttctgacacaactgtgttcactagcaacctcaaacagacacc

SEQ ID NO: 22 - DNA, 1653 bp, synthetic construct
  source 1..1653: mol_type = other DNA
atggaagacgccaaaaacattaagaagggcccagcgccattctacccactcgaagacgggaccgccggcgagcagctgcacaaagccatgaagcgctacgccctggtgcccggcaccatcgcctttaccgacgcacatatcgaggtggacattacctacgccgagtacttcgagatgagcgttcggctggcagaagctatgaagcgctatgggctgaatacaaaccatcggatcgtggtgtgcagcgagaatagcttgcagttcttcatgcccgtgttgggtgccctgttcatcggtgtggctgtggccccagctaacgacatctacaacgagcgcgagctgctgaacagcatgggcatcagccagcccaccgtcgtattcgtgagcaagaaagggctgcaaaagatcctcaacgtgcaaaagaagctaccgatcatacaaaagatcatcatcatggatagcaagaccgactaccagggcttccaaagcatgtacaccttcgtgacttcccatttgccacccggcttcaacgagtacgacttcgtgcccgagagcttcgaccgggacaaaaccatcgccctgatcatgaacagtagtggcagtaccggattgcccaagggcgtagccctaccgcaccgcaccgcttgtgtccgattcagtcatgcccgcgaccccatcttcggcaaccagatcatccccgacaccgctatcctcagcgtggtgccatttcaccacggcttcggcatgttcaccacgctgggctacttgatctgcggctttcgggtcgtgctcatgtaccgcttcgaggaggagctattcttgcgcagcttgcaagactataagattcaatctgccctgctggtgcccacactatttagcttcttcgctaagagcactctcatcgacaagtacgacctaagcaacttgcacgagatcgccagcggcggggcgccgctcagcaaggaggtaggtgaggccgtggccaaacgcttccacctaccaggcatccgccagggctacggcctgacagaaacaaccagcgccattctgatcacccccgaaggggacgacaagcctggcgcagtaggcaaggtggtgcccttcttcgaggctaaggtggtggacttggacaccggtaagacactgggtgtgaaccagcgcggcgagctgtgcgtccgtggccccatgatcatgagcggctacgttaacaaccccgaggctacaaacgctctcatcgacaaggacggctggctgcacagcggcgacatcgcctactgggacgaggacgagcacttcttcatcgtggaccggctcaaaagcctgatcaaatacaagggctaccaggtagccccagccgaactggagagcatcctgctgcaacaccccaacatcttcgacgccggggtcgccggcctgcccgacgacgatgccggcgagctgcccgccgcagtcgtcgtgctggaacacggtaaaaccatgaccgagaaggagatcgtggactatgtggccagccaggttacaaccgccaagaagctgcgcggtggtgttgtgttcgtggacgaggtgcctaaaggactgaccggcaagttggacgcccgcaagatccgcgagattctcattaaggccaagaagggcggaaagatcgccgtgtaa

SEQ ID NO: 23 - DNA, 2298 bp, synthetic construct
  source 1..2298: mol_type = other DNA
atggatgctatgaaacggggcctgtgctgcgtgctgctcctgtgcggcgctgtgtttgtgagccctagcatcacccaggactgctccttccaacacagccccatctcctccgacttcgctgtcaaaatccgtgagctgtctgactacctgcttcaagattacccagtcaccgtggcctccaacctgcaggacgaggagctctgcgggggcctctggcggctggtcctggcacagcgctggatggagcggctcaagactgtcgctgggtccaagatgcaaggcttgctggagcgcgtgaacacggagatacactttgtcaccaaatgtgcctttcagcccccccccagctgtcttcgcttcgtccagaccaacatctcccgcctcctgcaggagacctccgagcagctggtggcgctgaagccctggatcactcgccagaacttctcccggtgcctggagctgcagtgtcagcccgactcctcaaccctgccacccccatggagtccccggcccctggaggccacagccccgacagccccgggcggcggcagcggcgatatgcaccagaagagaaccgccatgttccaggaccctcaggagagacctaggaagctgcctcacctgtgtacagagctccagacaaccatccacgacatcatcctggagtgcgtgtactgtaagcagcagctgctgagaagagaggtgtacgacttcgccttcagagacctgtgcatcgtgtacagagacggcaacccttacgccgtgtgcgataagtgtctgaagttctattccaaaatctccgaatataggtacatgcacggcgacacccctaccctgcacgagtacatgctggacctccagcctgagaccacagacctgtactgctacgagcagctgaacgacagctctgaggaagaggacgagattgacggacctgctggccaggccgagcctgacagagcccactacaatatcgtgacattctgttgcaaatgcgactccacactggacaagtgcctgaagttctacagcaagatctctgagtacagatactactgctactctgtgtacggcaccacactggagcagcagtacaacaagcctctgtgcgacctcctgatccgctgcatcaactgccagaagcctctgtgccctgaggagaagcagagacacctggacaagaagcagcggttccacaacatcagaggcagatggaccggcaggtgcatgtcctgctgtagatcctccagaaccagacgggagacccagctgcactacaacatcgtgaccttctgctgcaagtgcgactctaccctgagactgtgcgtgcagtctacccacgtggacatcagaaccctggaggacctgctgatgggcaccctgggcatcgtgtgccctatctgctctcagaagcctatggccaggttcgaggaccctaccagaagaccctacaagctgcctgacctgtgcaccgagctgaacacctctctgcaagacatcgagatcacctgcgtgtactgcaagaccgtgctggagctgaccgaggtgttcgagttcgccttcaaggacctgttcgtggtgtacagagacagcatccctcacgctgcctgccacaagtgcatcgacttctattccaggatcagggagctgcgctattactccgactctgtgatgtacggccccaaggccaccctccaggacatcgtgctgcacctggagcctcagaacgagatccccgtggacctgctgtgccacgagcagctgtctgactctgaagaggagaacgacgagatcgacggcgtgaaccaccagcacctgcctgccaggagagctgaaccccagcggcataccatgctgtgtatgtgcttctactctaggatcagagagctgaggtactactctgactctgtgtacggcgacaccctggagaagctgaccaacaccggcctgtacaacctgctgatccggtgcctgaggtgccagaagcctctgaaccctgccgagaagctgagacacctgaacgagaagagaagattccacaagatcgctggccactacagaggccagtgccactcttgctgcaacagagccagacaggagagactccagcggagaagggagacccaggtggccaggagagccgagcctcagagacacaccatgctgtgcatgtgctgcaagtgcgaggccagaatcgagctggtggtggagagctctgccgacgacctgagagccttccagcagctgttcctgtctaccctgagcttcgtgtgcccttggtgcgcctctcagcagtaa

SEQ ID NO: 24 - DNA, 2711 bp, synthetic construct
  source 1..2711: mol_type = other DNA
acatttgcttctgacacaactgtgttcactagcaacctcaaacagacaccggatccgccaccatggatgctatgaaacggggcctgtgctgcgtgctgctcctgtgcggcgctgtgtttgtgagccctagcatcacccaggactgctccttccaacacagccccatctcctccgacttcgctgtcaaaatccgtgagctgtctgactacctgcttcaagattacccagtcaccgtggcctccaacctgcaggacgaggagctctgcgggggcctctggcggctggtcctggcacagcgctggatggagcggctcaagactgtcgctgggtccaagatgcaaggcttgctggagcgcgtgaacacggagatacactttgtcaccaaatgtgcctttcagcccccccccagctgtcttcgcttcgtccagaccaacatctcccgcctcctgcaggagacctccgagcagctggtggcgctgaagccctggatcactcgccagaacttctcccggtgcctggagctgcagtgtcagcccgactcctcaaccctgccacccccatggagtccccggcccctggaggccacagccccgacagccccgggcggcggcagcggcgatatgcaccagaagagaaccgccatgttccaggaccctcaggagagacctaggaagctgcctcacctgtgtacagagctccagacaaccatccacgacatcatcctggagtgcgtgtactgtaagcagcagctgctgagaagagaggtgtacgacttcgccttcagagacctgtgcatcgtgtacagagacggcaacccttacgccgtgtgcgataagtgtctgaagttctattccaaaatctccgaatataggtacatgcacggcgacacccctaccctgcacgagtacatgctggacctccagcctgagaccacagacctgtactgctacgagcagctgaacgacagctctgaggaagaggacgagattgacggacctgctggccaggccgagcctgacagagcccactacaatatcgtgacattctgttgcaaatgcgactccacactggacaagtgcctgaagttctacagcaagatctctgagtacagatactactgctactctgtgtacggcaccacactggagcagcagtacaacaagcctctgtgcgacctcctgatccgctgcatcaactgccagaagcctctgtgccctgaggagaagcagagacacctggacaagaagcagcggttccacaacatcagaggcagatggaccggcaggtgcatgtcctgctgtagatcctccagaaccagacgggagacccagctgcactacaacatcgtgaccttctgctgcaagtgcgactctaccctgagactgtgcgtgcagtctacccacgtggacatcagaaccctggaggacctgctgatgggcaccctgggcatcgtgtgccctatctgctctcagaagcctatggccaggttcgaggaccctaccagaagaccctacaagctgcctgacctgtgcaccgagctgaacacctctctgcaagacatcgagatcacctgcgtgtactgcaagaccgtgctggagctgaccgaggtgttcgagttcgccttcaaggacctgttcgtggtgtacagagacagcatccctcacgctgcctgccacaagtgcatcgacttctattccaggatcagggagctgcgctattactccgactctgtgatgtacggccccaaggccaccctccaggacatcgtgctgcacctggagcctcagaacgagatccccgtggacctgctgtgccacgagcagctgtctgactctgaagaggagaacgacgagatcgacggcgtgaaccaccagcacctgcctgccaggagagctgaaccccagcggcataccatgctgtgtatgtgcttctactctaggatcagagagctgaggtactactctgactctgtgtacggcgacaccctggagaagctgaccaacaccggcctgtacaacctgctgatccggtgcctgaggtgccagaagcctctgaaccctgccgagaagctgagacacctgaacgagaagagaagattccacaagatcgctggccactacagaggccagtgccactcttgctgcaacagagccagacaggagagactccagcggagaagggagacccaggtggccaggagagccgagcctcagagacacaccatgctgtgcatgtgctgcaagtgcgaggccagaatcgagctggtggtggagagctctgccgacgacctgagagccttccagcagctgttcctgtctaccctgagcttcgtgtgcccttggtgcgcctctcagcagtaaggcgcgccgctcgctttcttgctgtccaatttctattaaaggttcctttgttccctaagtccaactactaaactgggggatattatgaagggccttgagcatctggattctgcctgctcgctttcttgctgtccaatttctattaaaggttcctttgttccctaagtccaactactaaactgggggatattatgaagggccttgagcatctggattctgcctgaattcaaaaaaaaaaaaaaaaaaaaaaaaaaaaaaaaaaaaaaaaaaaaaaaaaaaaaaaaaaaagatatcaaaaaaaaaaaaaaaaaaagaaaaaaaaaaaaaaaaaaagaaaaaaaaaaaaaaaaa

SEQ ID NO: 25 - DNA, 2713 bp, synthetic construct
  source 1..2713: mol_type = other DNA
acatttgcttctgacacaactgtgttcactagcaacctcaaacagacaccggatccgccaccatggatgctatgaaacggggcctgtgctgcgtgctgctcctgtgcggcgctgtgtttgtgagccctagcatcacccaggactgctccttccaacacagccccatctcctccgacttcgctgtcaaaatccgtgagctgtctgactacctgcttcaagattacccagtcaccgtggcctccaacctgcaggacgaggagctctgcgggggcctctggcggctggtcctggcacagcgctggatggagcggctcaagactgtcgctgggtccaagatgcaaggcttgctggagcgcgtgaacacggagatacactttgtcaccaaatgtgcctttcagcccccccccagctgtcttcgcttcgtccagaccaacatctcccgcctcctgcaggagacctccgagcagctggtggcgctgaagccctggatcactcgccagaacttctcccggtgcctggagctgcagtgtcagcccgactcctcaaccctgccacccccatggagtccccggcccctggaggccacagccccgacagccccgggcggcggcagcggcgatatgcaccagaagagaaccgccatgttccaggaccctcaggagagacctaggaagctgcctcacctgtgtacagagctccagacaaccatccacgacatcatcctggagtgcgtgtactgtaagcagcagctgctgagaagagaggtgtacgacttcgccttcagagacctgtgcatcgtgtacagagacggcaacccttacgccgtgtgcgataagtgtctgaagttctattccaaaatctccgaatataggtacatgcacggcgacacccctaccctgcacgagtacatgctggacctccagcctgagaccacagacctgtactgctacgagcagctgaacgacagctctgaggaagaggacgagattgacggacctgctggccaggccgagcctgacagagcccactacaatatcgtgacattctgttgcaaatgcgactccacactggacaagtgcctgaagttctacagcaagatctctgagtacagatactactgctactctgtgtacggcaccacactggagcagcagtacaacaagcctctgtgcgacctcctgatccgctgcatcaactgccagaagcctctgtgccctgaggagaagcagagacacctggacaagaagcagcggttccacaacatcagaggcagatggaccggcaggtgcatgtcctgctgtagatcctccagaaccagacgggagacccagctgcactacaacatcgtgaccttctgctgcaagtgcgactctaccctgagactgtgcgtgcagtctacccacgtggacatcagaaccctggaggacctgctgatgggcaccctgggcatcgtgtgccctatctgctctcagaagcctatggccaggttcgaggaccctaccagaagaccctacaagctgcctgacctgtgcaccgagctgaacacctctctgcaagacatcgagatcacctgcgtgtactgcaagaccgtgctggagctgaccgaggtgttcgagttcgccttcaaggacctgttcgtggtgtacagagacagcatccctcacgctgcctgccacaagtgcatcgacttctattccaggatcagggagctgcgctattactccgactctgtgatgtacggccccaaggccaccctccaggacatcgtgctgcacctggagcctcagaacgagatccccgtggacctgctgtgccacgagcagctgtctgactctgaagaggagaacgacgagatcgacggcgtgaaccaccagcacctgcctgccaggagagctgaaccccagcggcataccatgctgtgtatgtgcttctactctaggatcagagagctgaggtactactctgactctgtgtacggcgacaccctggagaagctgaccaacaccggcctgtacaacctgctgatccggtgcctgaggtgccagaagcctctgaaccctgccgagaagctgagacacctgaacgagaagagaagattccacaagatcgctggccactacagaggccagtgccactcttgctgcaacagagccagacaggagagactccagcggagaagggagacccaggtggccaggagagccgagcctcagagacacaccatgctgtgcatgtgctgcaagtgcgaggccagaatcgagctggtggtggagagctctgccgacgacctgagagccttccagcagctgttcctgtctaccctgagcttcgtgtgcccttggtgcgcctctcagcagtaaggcgcgccgctcgctttcttgctgtccaatttctattaaaggttcctttgttccctaagtccaactactaaactgggggatattatgaagggccttgagcatctggattctgcctgctcgctttcttgctgtccaatttctattaaaggttcctttgttccctaagtccaactactaaactgggggatattatgaagggccttgagcatctggattctgcctgaattcaaaaaaaaaaaaaaaaaaagaaaaaaaaaaaaaaaaaaagaaaaaaaaaaaaaaaaaaagatatcaaaaaaaaaaaaaaaaaaaaaaaaaaaaaaaaaaaaaaaaaaaaaaaaaaaaaaaaaaaa

SEQ ID NO: 26 - protein, 765 aa, synthetic construct
MDAMKRGLCCVLLLCGAVFVSPSITQDCSFQHSPISSDFAVKIRELSDYLLQDYPVTVASNLQDEELCGGLWRLVLAQRWMERLKTVAGSKMQGLLERVNTEIHFVTKCAFQPPPSCLRFVQTNISRLLQETSEQLVALKPWITRQNFSRCLELQCQPDSSTLPPPWSPRPLEATAPTAPGGGSGDMHQKRTAMFQDPQERPRKLPHLCTELQTTIHDIILECVYCKQQLLRREVYDFAFRDLCIVYRDGNPYAVCDKCLKFYSKISEYRYMHGDTPTLHEYMLDLQPETTDLYCYEQLNDSSEEEDEIDGPAGQAEPDRAHYNIVTFCCKCDSTLDKCLKFYSKISEYRYYCYSVYGTTLEQQYNKPLCDLLIRCINCQKPLCPEEKQRHLDKKQRFHNIRGRWTGRCMSCCRSSRTRRETQLHYNIVTFCCKCDSTLRLCVQSTHVDIRTLEDLLMGTLGIVCPICSQKPMARFEDPTRRPYKLPDLCTELNTSLQDIEITCVYCKTVLELTEVFEFAFKDLFVVYRDSIPHAACHKCIDFYSRIRELRYYSDSVMYGPKATLQDIVLHLEPQNEIPVDLLCHEQLSDSEEENDEIDGVNHQHLPARRAEPQRHTMLCMCFYSRIRELRYYSDSVYGDTLEKLTNTGLYNLLIRCLRCQKPLNPAEKLRHLNEKRRFHKIAGHYRGQCHSCCNRARQERLQRRRETQVARRAEPQRHTMLCMCCKCEARIELVVESSADDLRAFQQLFLSTLSFVCPWCASQQ